European Patent Application EP 4 343 328 A2, published March 27, 2024. Title: Sposób i kompozycja diagnostyczna do wykrywania mastitis. Applicant: Uniwersytet Jagielloński. Application EP. The sequence listing filed with the application follows.

SEQUENCE LISTING (51 sequences)

SEQ ID NO: 1 - protein, 346 aa, Escherichia coli
MKKTAIAIAVALAGFATVAQAAPKDNTWYTGAKLGWSQYHDTGFINNNGPTHENQLGAGAFGGYQVNPYVGFEMGYDWLGRMPYKGSVENGAYKAQGVQLTAKLGYPITDDLDIYTRLGGMVWRADTKSNVYGKNHDTGVSPVFAGGVEYAITPEIATRLEYQWTNNIGDAHTIGTRPDNGMLSLGVSYRFGQGEAAPVVAPAPAPAPEVQTKHFTLKSDVLFNFNKATLKPEGQAALDQLYSQLSNLDPKDGSVVVLGYTDRIGSDAYNQGLSERRAQSVVDYLISKGIPADKISARGMGESNPVTGNTCDNVKQRAALIDCLAPDRRVEIEVKGIKDVVTQPQA

SEQ ID NO: 2 - protein, 398 aa, Streptococcus uberis
MAKEKYDRSKPHVNIGTIGHVDHGKTTLTAAITTVLARRLPTSVNQPKDYASIDAAPEERERGITINTAHVEYETETRHYAHIDAPGHADYVKNMITGAAQMDGAILVVASTDGPMPQTREHILLSRQVGVKHLIVFMNKIDLVDDEELLELVEMEIRDLLSEYDFPGDDLPVIQGSALKALEGDSKYEDIIMELMKTADEYIPEPERDTDKPLLLPVEDVFSITGRGTVASGRIDRGTVRVNDEIEIVGIKEETKKAVVTGVEMFRKQLDEGLAGDNVGILLRGVQRDEIERGQVIAKPGSINPHTKFKGEVYILSKDEGGRHTPFFNNYRPQFYFRTTDVTGSIELPAGTEMVMPGDNVTISVELIHPIAVEQGTTFSIREGGRTVGSGIVSEIEA

SEQ ID NO: 3 - protein, 340 aa, Streptococcus agalactiae
MTQAVLKELAKAELHCHLDGSLSLPAIRKLANMADIILPSSDKELRKYVIAPAQTESLVDYLKTFEFIRPLLQTKEALRFAAYDVARQAALENVIYIEIRFAPELSMDKGLTASDTVLAVLEGLADAQKEFNIVARALVCGMRQSSHKTTKDIIKHIVDLAPKGLVGFDFAGDEFSYPTDSLVDLIQEVKRSGYPMTLHAGECGCAKHIADSLNLGIKRMGHVTALTGQRDLIKRFVEEDVVAEMCLTSNLQTKAASSIQSFPYQELYDAGGKITINTDNRTVSDTNLTKEYSLFVTYFGTKIEDFLVFNQNAVKASFTSDSEKDTLLHKLQENYDSYLK

SEQ ID NO: 4 - protein, 1103 aa, Staphylococcus aureus
MKNSLRYGIRKHKLGAASVFLGTMIVVGMGQDKEAAASEQNTTVEENGNSATENKSKQTTTNNVNNIDETQTYSATSTEQPSNATQVTAEAAPQAVEAPQTSQAPQKVQSTNVETVKEEVVKEEVQPQVKETARSQENSGDQRQVDLTPKKVTQNQGTEPQVEVAQPRTVSESKPRVTRSTDVAEAKDASEIKGTDVTSKVTVESGSIEAPQGNKVEPHAGQRVVLKYKLKFEKGLHKDDYFDFTLSNNVNTHGVSTARKVPDIKNGTVVMATGQLLGNGKIRYTFTDYIDYKVNVTADLEINLFIDPKTVQSNGQQIITSTLNDKETRTTLPIQYNPGVSNSYANVNGSIETFDKGNNKFTHVAYIKPQNGHKSDSVSITGTLTQGSKANGNAPTVKVYEVLKDAKELPESVYANISDSTMFKDVTQEMKDKLKVENNGSYKLDIEKLEKSYVIHYDGEYLSGSDQVNFRTHMFGYPEQQYKYYYTHLGYQLTWDNGLVLYSNKAKGDGTNGTITESNNMTFDEEYGNGVITGQYDKNLVTTVEEEYDSSTLDIDYHTAIDGEGGYVDGYIETIEETDSSAIDIDYHTAVDSEAGHVGGYTESSEESNPIDFEESTHENSKHHADVVEYEEDTNPGGGQVTTESNLLEFDEESTKGIVTGAISDHTTVEDTKEYTTESNLIELVDELPEEHGQAQGPIEEITENNQHISHSGLGTENGHGNYGIVEEIEENSHVDIKSELGYEGGQNIGNQSFEEDTEEDKPKYEQGGNIVDIDFDSVPQIQGQNKGDQSFEEDTEEDKPKYEQGGNIVDIDFDSVPQIQGQNKGNQSFEEDTEKDKPKYEHGGNIIDIDFDSVPHIHGFNKHTEIIEEDTNKDKPSYQFGGHNSVDFEEDTLPQVSGQNEGQQTIEEDTTPPIVPPTPPTPEVPSEPETPTPPTPEVPSEPETPTPTPPTPEVPSEPETPTPPTPEVPSEPETPTPTPPTPEVPSEPETPTPPTPEVPSEPETPTPPMPEIPAEPGKPVPPANEEPKKPSKPVEQGKVVTPVIEINEKVKAVKPAKTSQSKKTELPETGGEETTNNGVLFGGLLSIIGLVLLRRNKKNHKA

SEQ ID NO: 5 - protein, 24 aa, synthetic construct
  REGION 1..24: note = epitop
WSQYHDTGFINNNGPTHENQLGAG

SEQ ID NO: 6 - protein, 18 aa, synthetic construct
  REGION 1..18: note = epitop
YDWLGRMPYKGSVENGAY

SEQ ID NO: 7 - protein, 6 aa, synthetic construct
  REGION 1..6: note = epitop
GYPITD

SEQ ID NO: 8 - protein, 17 aa, synthetic construct
  REGION 1..17: note = epitop
DTKSNVYGKNHDTGVSP

SEQ ID NO: 9 - protein, 61 aa, synthetic construct
  REGION 1..61: note = epitop
EIATRLEYQWTNNIGDAHTIGTRPDNGMLSLGVSYRFGQGEAAPVVAPAPAPAPEVQTKHF

SEQ ID NO: 10 - protein, 12 aa, synthetic construct
  REGION 1..12: note = epitop
LFNFNKATLKPE

SEQ ID NO: 11 - protein, 13 aa, synthetic construct
  REGION 1..13: note = epitop
IGSDAYNQGLSER

SEQ ID NO: 12 - protein, 24 aa, synthetic construct
  REGION 1..24: note = epitop
ESNPVTGNTCDNVKQRAALIDCLA

SEQ ID NO: 13 - protein, 6 aa, synthetic construct
  REGION 1..6: note = epitop
IKDVVT

SEQ ID NO: 14 - protein, 7 aa, synthetic construct
  REGION 1..7: note = epitop
EKYDRSK

SEQ ID NO: 15 - protein, 26 aa, synthetic construct
  REGION 1..26: note = epitop
ARRLPTSVNQPKDYASIDAAPEERER

SEQ ID NO: 16 - protein, 8 aa, synthetic construct
  REGION 1..8: note = epitop
VDDEELLE

SEQ ID NO: 17 - protein, 5 aa, synthetic construct
  REGION 1..5: note = epitop
DFPGD

SEQ ID NO: 18 - protein, 11 aa, synthetic construct
  REGION 1..11: note = epitop
ALEGDSKYEDI

SEQ ID NO: 19 - protein, 10 aa, synthetic construct
  REGION 1..10: note = epitop
EYIPEPERDT

SEQ ID NO: 20 - protein, 11 aa, synthetic construct
  REGION 1..11: note = epitop
EMFRKQLDEGL

SEQ ID NO: 21 - protein, 7 aa, synthetic construct
  REGION 1..7: note = epitop
VQRDEIE

SEQ ID NO: 22 - protein, 12 aa, synthetic construct
  REGION 1..12: note = epitop
PGSINPHTKFKG

SEQ ID NO: 23 - protein, 14 aa, synthetic construct
  REGION 1..14: note = epitop
SKDEGGRHTPFFNN

SEQ ID NO: 24 - protein, 7 aa, synthetic construct
  REGION 1..7: note = epitop
AGTEMVM

SEQ ID NO: 25 - protein, 25 aa, synthetic construct
  REGION 1..25: note = epitop
IILPSSDKELRKYVIAPAQTESLVD

SEQ ID NO: 26 - protein, 9 aa, synthetic construct
  REGION 1..9: note = epitop
LSMDKGLTA

SEQ ID NO: 27 - protein, 7 aa, synthetic construct
  REGION 1..7: note = epitop
SSHKTTK

SEQ ID NO: 28 - protein, 8 aa, synthetic construct
  REGION 1..8: note = epitop
EFSYPTDS

SEQ ID NO: 29 - protein, 5 aa, synthetic construct
  REGION 1..5: note = epitop
TGQRD

SEQ ID NO: 30 - protein, 10 aa, synthetic construct
  REGION 1..10: note = epitop
TKAASSIQSF

SEQ ID NO: 31 - protein, 4 aa, synthetic construct
  REGION 1..4: note = epitop
TKIE

SEQ ID NO: 32 - protein, 18 aa, synthetic construct
  REGION 1..18: note = epitop
TSDSEKDTLLHKLQENYD

SEQ ID NO: 33 - protein, 10 aa, synthetic construct
  REGION 1..10: note = epitop
TDVTSKVTVE

SEQ ID NO: 34 - protein, 13 aa, synthetic construct
  REGION 1..13: note = epitop
IKPNNGKTTSVTV

SEQ ID NO: 35 - protein, 15 aa, synthetic construct
  REGION 1..15: note = epitop
KFENGLHQGDYFDFT

SEQ ID NO: 36 - protein, 6 aa, synthetic construct
  REGION 1..6: note = epitop
GNYYAN

SEQ ID NO: 37 - protein, 26 aa, synthetic construct
  REGION 1..26: note = epitop
ANTTDTSKFKEVTSNMSGNLNLQNNG

SEQ ID NO: 38 - protein, 12 aa, synthetic construct
  REGION 1..12: note = epitop
SLNIENLDKTYV

SEQ ID NO: 39 - protein, 23 aa, synthetic construct
  REGION 1..23: note = epitop
SNQNGNQPKVRIFEYLGNNEDIA

SEQ ID NO: 40 - protein, 22 aa, synthetic construct
  REGION 1..22: note = epitop
EVLEGGKIRYTFTNDIEDKVDV

SEQ ID NO: 41 - protein, 23 aa, synthetic construct
  REGION 1..23: note = epitop
VQTNGNQTITSTLNEEQTSKELD

SEQ ID NO: 42 - protein, 8 aa, synthetic construct
  REGION 1..8: note = epitop
TDVTSKVT

SEQ ID NO: 43 - protein, 15 aa, synthetic construct
  REGION 1..15: note = epitop
KFENGLHQGDYFDFT

SEQ ID NO: 44 - protein, 38 aa, synthetic construct
  REGION 1..38: note = epitop
ANTTDTSKFKEVTSNMNLNLQNNGSYSLNIENLDKTYV

SEQ ID NO: 45 - protein, 14 aa, synthetic construct
  REGION 1..14: note = epotop
IKPNNGKTTSVTVT

SEQ ID NO: 46 - protein, 7 aa, synthetic construct
  REGION 1..7: note = eopitop
MVGHPYT

SEQ ID NO: 47 - protein, 24 aa, synthetic construct
  REGION 1..24: note = epitop
GSNQNGNQPKVRIFEYLGNNEDIA

SEQ ID NO: 48 - protein, 31 aa, synthetic construct
  REGION 1..31: note = epitop
NGSVVMATGEVLEGGKIRYTFTNDIEDKVDV

SEQ ID NO: 49 - protein, 5 aa, synthetic construct
  REGION 1..5: note = epitop
GNYYA

SEQ ID NO: 50 - protein, 8 aa, synthetic construct
  REGION 1..8: note = epitop
DGEYLNGT

SEQ ID NO: 51 - protein, 5 aa, synthetic construct
  REGION 1..5: note = epitop
KANNR